European Patent Application EP 4 218 814 A2, published August 2, 2023. Title: Stabilized Formulations Containing Anti-PCSK9 Antibodies. Applicant: Regeneron Pharmaceuticals, Inc. Application EP. The sequence listing filed with the application follows.

SEQUENCE LISTING (9 sequences)

SEQ ID NO: 1 - protein, 118 aa, synthetic construct [sequence omitted]

SEQ ID NO: 2 - protein, 8 aa, synthetic construct
GFTFNNYA

SEQ ID NO: 3 - protein, 8 aa, synthetic construct
ISGSGGTT

SEQ ID NO: 4 - protein, 11 aa, synthetic construct
AKDSNWGNFDL

SEQ ID NO: 5 - protein, 113 aa, synthetic construct [sequence omitted]

SEQ ID NO: 6 - protein, 12 aa, synthetic construct
QSVLYRSNNRNF

SEQ ID NO: 7 - skipped

SEQ ID NO: 8 - protein, 9 aa, synthetic construct
QQYYTTPYT

SEQ ID NO: 9 - protein, 692 aa, synthetic construct
MGTVSSRRSWWPLPLPLLLLLLLGPAGARAQEDEDGDYEELVLALRSEEDGLADAPEHGATATFHRCAKDPWRLPGTYVVVLKEETHRSQSERTARRLQAQAARRGYLTKILHVFHHLLPGFLVKMSGDLLELALKLPHVDYIEEDSSVFAQSIPWNLERITPARYRADEYQPPKGGSLVEVYLLDTSIQSDHREIEGRVMVTDFESVPEEDGTRFHRQASKCDSHGTHLAGVVSGRDAGVAKGAGLRSLRVLNCQGKGTVSGTLIGLEFIRKSQLVQPVGPLVVLLPLAGGYSRVFNAACQRLARAGVVLVTAAGNFRDDACLYSPASAPEVITVGATNAQDQPVTLGTLGTNFGRCVDLFAPGEDIIGASSDCSTCFVSRSGTSQAAAHVAGIAAMMLSAEPELTLAELRQRLIHFSAKDVINEAWFPEDQRVLTPNLVAALPPSTHRAGWQLFCRTVWSAHSGPTRMATAVARCAQDEELLSCSSFSRSGKRRGERIEAQGGKRVCRAHNAFGGEGVYAIARCCLLPQVNCSVHTAPPAGASMGTRVHCHQQGHVLTGCSSHWEVEDLGTHKPPVLRPRGQPNQCVGHREASIHASCCHAPGLECKVKEHGIPAPQEQVIVACEDGWTLTGCSPLPGTSHVLGAYAVDNTCVVRSRDVSTTGSTSKEAVAAVAICCRSRHLVQASQELQ